European Patent Application EP 4 624 493 A1, published October 1, 2025. Title: PHARMACEUTICAL COMPOSITION COMPRISING BISPECIFIC ANTIBODY SPECIFICALLY BINDING TO HGFR AND EGFR. Applicant: JIANGSU HENGRUI PHARMACEUTICALS CO., LTD. Application IB PCT/CN2023/133895, filed November 24, 2023. The sequence listing filed with the application follows.

SEQUENCE LISTING (51 sequences)

SEQ ID NO: 1 - protein, 455 aa, synthetic construct
QVQLVESGGGVVQPGRSLRLSCAASGFTFSTYGMHWVRQAPGKGLEWVAVIWDDGSYKYYGDSVKGRFTISRDNSKNTLYLQMNSLRAEDTAVYYCARDGITMVRGVMKDYFDYWGQGTLVTVSSASTKGPSVFPLAPSSKSTSGGTAALGCLVKDYFPEPVTVSWNSGALTSGVHTFPAVLQSSGLYSLSSVVTVPSSSLGTQTYICNVNHKPSNTKVDKRVEPKSCDKTHTCPPCPAPELLGGPSVFLFPPKPKDTLMISRTPEVTCVVVDVSHEDPEVKFNWYVDGVEVHNAKTKPREEQYNSTYRVVSVLTVLHQDWLNGKEYKCKVSNKALPAPIEKTISKAKGQPREPQVYTLPPSREEMTKNQVSLTCLVKGFYPSDIAVEWESNGQPENNYKTTPPVLDSDGSFFLYSKLTVDKSRWQQGNVFSCSVMHEALHNHYTQKSLSLSPGK

SEQ ID NO: 2 - protein, 214 aa, synthetic construct
AIQLTQSPSSLSASVGDRVTITCRASQDISSALVWYQQKPGKAPKLLIYDASSLESGVPSRFSGSESGTDFTLTISSLQPEDFATYYCQQFNSYPLTFGGGTKVEIKRTVAAPSVFIFPPSDEQLKSGTASVVCLLNNFYPREAKVQWKVDNALQSGNSQESVTEQDSKDSTYSLSSTLTLSKADYEKHKVYACEVTHQGLSSPVTKSFNRGEC

SEQ ID NO: 3 - protein, 125 aa, synthetic construct [sequence omitted]

SEQ ID NO: 4 - protein, 107 aa, synthetic construct [sequence omitted]

SEQ ID NO: 5 - protein, 107 aa, synthetic construct
DIQLTQSPSSLSASVGDRVTITCRASQDISSALVWYQQKPGKAPKLLIYDASSLESGVPSRFSGSESGTDFTLTISSLQPEDFATYYCQQFNSYPLTFGGGTKVEIK

SEQ ID NO: 6 - protein, 5 aa, synthetic construct
TYGMH

SEQ ID NO: 7 - protein, 17 aa, synthetic construct
VIWDDGSYKYYGDSVKG

SEQ ID NO: 8 - protein, 16 aa, synthetic construct
DGITMVRGVMKDYFDY

SEQ ID NO: 9 - protein, 11 aa, synthetic construct
RASQDISSALV

SEQ ID NO: 10 - protein, 7 aa, synthetic construct
DASSLES

SEQ ID NO: 11 - protein, 9 aa, synthetic construct
QQFNSYPLT

SEQ ID NO: 12 - protein, 119 aa, synthetic construct [sequence omitted]

SEQ ID NO: 13 - protein, 113 aa, synthetic construct [sequence omitted]

SEQ ID NO: 14 - protein, 120 aa, synthetic construct
QVQLVESGGGVVQPGRSLRLSCAASGFSLSNYGVHWVRQAPGKGLEWLAVIWSGGSTNYAAAFVSRLTISKDNSKNTVYLQMNSLRAEDTAVYYCARNHDNPYNYAMDYWGQGTTVTVSS

SEQ ID NO: 15 - protein, 111 aa, synthetic construct
DIVLTQSPDSLAVSLGERATINCRADKSVSTSTYNYLHWYQQKPGQPPKLLIYLASNLASGVPDRFSGSGSGTDFTLTISSLQAEDVAVYYCQHSRDLPPTFGQGTKLEIK

SEQ ID NO: 16 - protein, 120 aa, synthetic construct
QVQLVESGGGVVQPGRSLRLSCAASGFSLSDYGVHWVRQAPGKGLEWLAVIWSGGSTNYADAFVSRLTISKDNSKNTVYLQMNSLRAEDTAVYYCARNHDNPYIYAMDYWGQGTTVTVSS

SEQ ID NO: 17 - protein, 111 aa, synthetic construct
DIVLTQSPDSLAVSLGERATINCRADKSVSTSTYNYLHWYQQKPGQPPKLLIYRGSFLATGVPDRFSGSGSGTDFTLTISSLQAEDVAVYYCQHSRDLPPTFGQGTKLEIK

SEQ ID NO: 18 - protein, 5 aa, synthetic construct
SYWLH

SEQ ID NO: 19 - protein, 17 aa, synthetic construct
MIDPSNSDTRFNPNFKD

SEQ ID NO: 20 - protein, 10 aa, synthetic construct
YRSYVTPLDY

SEQ ID NO: 21 - protein, 17 aa, synthetic construct
KSSQSLLYTSSQKNYLA

SEQ ID NO: 22 - protein, 7 aa, synthetic construct
WASTRES

SEQ ID NO: 23 - protein, 9 aa, synthetic construct
QQYYAYPWT

SEQ ID NO: 24 - protein, 5 aa, synthetic construct
NYGVH

SEQ ID NO: 25 - protein, 16 aa, synthetic construct
VIWSGGSTNYAAAFVS

SEQ ID NO: 26 - protein, 12 aa, synthetic construct
NHDNPYNYAMDY

SEQ ID NO: 27 - protein, 15 aa, synthetic construct
RADKSVSTSTYNYLH

SEQ ID NO: 28 - protein, 7 aa, synthetic construct
LASNLAS

SEQ ID NO: 29 - protein, 9 aa, synthetic construct
QHSRDLPPT

SEQ ID NO: 30 - protein, 5 aa, synthetic construct
DYGVH

SEQ ID NO: 31 - protein, 16 aa, synthetic construct
VIWSGGSTNYADAFVS

SEQ ID NO: 32 - protein, 12 aa, synthetic construct
NHDNPYIYAMDY

SEQ ID NO: 33 - protein, 7 aa, synthetic construct
RGSFLAT

SEQ ID NO: 34 - protein, 584 aa, synthetic construct
QVQLVESGGGVVQPGRSLRLSCAASGFTFSTYGMHWVRQAPGKGLEWVAVIWDDGSYKYYGDSVKGRFTISRDNSKNTLYLQMNSLRAEDTAVYYCARDGITMVRGVMKDYFDYWGQGTLVTVSSGGGGSGGGGQVQLVESGGGVVQPGRSLRLSCAASGFSLSDYGVHWVRQAPGKGLEWLAVIWSGGSTNYADAFVSRLTISKDNSKNTVYLQMNSLRAEDTAVYYCARNHDNPYIYAMDYWGQGTTVTVSSASTKGPSVFPLAPSSKSTSGGTAALGCLVKDYFPEPVTVSWNSGALTSGVHTFPAVLQSSGLYSLSSVVTVPSSSLGTQTYICNVNHKPSNTKVDKKVEPKSCDKTHTCPPCPAPELLGGPSVFLFPPKPKDTLMISRTPEVTCVVVDVSHEDPEVKFNWYVDGVEVHNAKTKPREEQYNSTYRVVSVLTVLHQDWLNGKEYKCKVSNKALPAPIEKTISKAKGQPREPQVYTLPPCREEMTKNQVSLWCLVKGFYPSDIAVEWESNGQPENNYKTTPPVLDSDGSFFLYSKLTVDKSRWQQGNVFSCSVMHEALHNHYTQKSLSLSPGK

SEQ ID NO: 35 - protein, 334 aa, synthetic construct
DIQLTQSPSSLSASVGDRVTITCRASQDISSALVWYQQKPGKAPKLLIYDASSLESGVPSRFSGSESGTDFTLTISSLQPEDFATYYCQQFNSYPLTFGGGTKVEIKGGGGSGGGGDIVLTQSPDSLAVSLGERATINCRADKSVSTSTYNYLHWYQQKPGQPPKLLIYRGSFLATGVPDRFSGSGSGTDFTLTISSLQAEDVAVYYCQHSRDLPPTFGQGTKLEIKRTVAAPSVFIFPPSDEQLKSGTASVVCLLNNFYPREAKVQWKVDNALQSGNSQESVTEQDSKDSTYSLSSTLTLSKADYEKHKVYACEVTHQGLSSPVTKSFNRGEC

SEQ ID NO: 36 - protein, 449 aa, synthetic construct
EVQLVESGGGLVQPGGSLRLSCAASGYTFTSYWLHWVRQAPGKGLEWVGMIDPSNSDTRFNPNFKDRFTISADTSKNTAYLQMNSLRAEDTAVYYCATYRSYVTPLDYWGQGTLVTVSSGGGGSGIPPKIECLPIDISIDEGKVLTVASAFTGEPTPEVTWSTGGRKIHSQEQGRFHIENTDDSTTLTIKDVQKQDGGLYTLTLRNEFGSDSATVNIHIRSIDKTHTCPPCPAPELLGGPSVFLFPPKPKDTLMISRTPEVTCVVVDVSHEDPEVKFNWYVDGVEVHNAKTKPREEQYNSTYRVVSVLTVLHQDWLNGKEYKCKVSNKALPAPIEKTISKAKGQPREPQVCTLPPSREEMTKNQVSLSCAVKGFYPSDIAVEWESNGQPENNYKTTPPVLDSDGSFFLVSKLTVDKSRWQQGNVFSCSVMHEALHNHYTQKSLSLSPGK

SEQ ID NO: 37 - protein, 215 aa, synthetic construct
DIQMTQSPSSLSASVGDRVTITCKSSQSLLYTSSQKNYLAWYQQKPGKAPKLLIYWASTRESGVPSRFSGSGSGTDFTLTISSLQPEDFATYYCQQYYAYPWTFGQGTKVEIKGGGGSSGAPRFLTRPKASVVSVGKDATLSCQIVGNPFPQVSWEKDKQPVTAGVRFRLAQDGDLYRLKILDLQLSDSGQYVCRARNAHGEAFACLGLQVDAEA

SEQ ID NO: 38 - protein, 449 aa, synthetic construct
EVQLVESGGGLVQPGGSLRLSCAASGYTFTSYWLHWVRQAPGKGLEWVGMIDPSNSDTRFNPNFKDRFTISADTSKNTAYLQMNSLRAEDTAVYYCATYRSYVTPLDYWGQGTLVTVSSASTKGPSVFPLAPSSKSTSGGTAALGCLVKDYFPEPVTVSWNSGALTSGVHTFPAVLQSSGLYSLSSVVTVPSSSLGTQTYICNVNHKPSNTKVDKKVEPKSCDKTHTCPPCPAPELLGGPSVFLFPPKPKDTLMISRTPEVTCVVVDVSHEDPEVKFNWYVDGVEVHNAKTKPREEQYNSTYRVVSVLTVLHQDWLNGKEYKCKVSNKALPAPIEKTISKAKGQPREPQVYTLPPCREEMTKNQVSLWCLVKGFYPSDIAVEWESNGQPENNYKTTPPVLDSDGSFFLYSKLTVDKSRWQQGNVFSCSVMHEALHNHYTQKSLSLSPGK

SEQ ID NO: 39 - protein, 220 aa, synthetic construct
DIQMTQSPSSLSASVGDRVTITCKSSQSLLYTSSQKNYLAWYQQKPGKAPKLLIYWASTRESGVPSRFSGSGSGTDFTLTISSLQPEDFATYYCQQYYAYPWTFGQGTKVEIKRTVAAPSVFIFPPSDEQLKSGTASVVCLLNNFYPREAKVQWKVDNALQSGNSQESVTEQDSKDSTYSLSSTLTLSKADYEKHKVYACEVTHQGLSSPVTKSFNRGEC

SEQ ID NO: 40 - protein, 455 aa, synthetic construct
QVQLVESGGGVVQPGRSLRLSCAASGFTFSTYGMHWVRQAPGKGLEWVAVIWDDGSYKYYGDSVKGRFTISRDNSKNTLYLQMNSLRAEDTAVYYCARDGITMVRGVMKDYFDYWGQGTLVTVSSGGGGSGIPPKIECLPIDISIDEGKVLTVASAFTGEPTPEVTWSTGGRKIHSQEQGRFHIENTDDSTTLTIKDVQKQDGGLYTLTLRNEFGSDSATVNIHIRSIDKTHTCPPCPAPELLGGPSVFLFPPKPKDTLMISRTPEVTCVVVDVSHEDPEVKFNWYVDGVEVHNAKTKPREEQYNSTYRVVSVLTVLHQDWLNGKEYKCKVSNKALPAPIEKTISKAKGQPREPQVCTLPPSREEMTKNQVSLSCAVKGFYPSDIAVEWESNGQPENNYKTTPPVLDSDGSFFLVSKLTVDKSRWQQGNVFSCSVMHEALHNHYTQKSLSLSPGK

SEQ ID NO: 41 - protein, 209 aa, synthetic construct
DIQLTQSPSSLSASVGDRVTITCRASQDISSALVWYQQKPGKAPKLLIYDASSLESGVPSRFSGSESGTDFTLTISSLQPEDFATYYCQQFNSYPLTFGGGTKVEIKGGGGSSGAPRFLTRPKASVVSVGKDATLSCQIVGNPFPQVSWEKDKQPVTAGVRFRLAQDGDLYRLKILDLQLSDSGQYVCRARNAHGEAFACLGLQVDAEA

SEQ ID NO: 42 - protein, 627 aa, synthetic construct
LEEKKVCQGTSNKLTQLGTFEDHFLSLQRMFNNCEVVLGNLEITYVQRNYDLSFLKTIQEVAGYVLIALNTVERIPLENLQIIRGNMYYENSYALAVLSNYDANKTGLKELPMRNLQEILHGAVRFSNNPALCNVESIQWRDIVSSDFLSNMSMDFQNHLGSCQKCDPSCPNGSCWGAGEENCQKLTKIICAQQCSGRCRGKSPSDCCHNQCAAGCTGPRESDCLVCRKFRDEATCKDTCPPLMLYNPTTYQMDVNPEGKYSFGATCVKKCPRNYVVTDHGSCVRACGADSYEMEEDGVRKCKKCEGPCRKVCNGIGIGEFKDSLSINATNIKHFKNCTSISGDLHILPVAFRGDSFTHTPPLDPQELDILKTVKEITGFLLIQAWPENRTDLHAFENLEIIRGRTKQHGQFSLAVVSLNITSLGLRSLKEISDGDVIISGNKNLCYANTINWKKLFGTSGQKTKIISNRGENSCKATGQVCHALCSPEGCWGPEPRDCVSCRNVSRGRECVDKCNLLEGEPREFVENSECIQCHPECLPQAMNITCTGRGPDNCIQCAHYIDGPHCVKTCPAGVMGENNTLVWKYADAGHVCHLCHPNCTYGCTGPGLEGCPTNGPKIPSHHHHHH

SEQ ID NO: 43 - protein, 914 aa, synthetic construct
ECKEALAKSEMNVNMKYQLPNFTAETPIQNVILHEHHIFLGATNYIYVLNEEDLQKVAEYKTGPVLEHPDCFPCQDCSSKANLSGGVWKDNINMALVVDTYYDDQLISCGSVNRGTCQRHVFPHNHTADIQSEVHCIFSPQIEEPSQCPDCVVSALGAKVLSSVKDRFINFFVGNTINSSYFPDHPLHSISVRRLKETKDGFMFLTDQSYIDVLPEFRDSYPIKYVHAFESNNFIYFLTVQRETLDAQTFHTRIIRFCSINSGLHSYMEMPLECILTEKRKKRSTKKEVFNILQAAYVSKPGAQLARQIGASLNDDILFGVFAQSKPDSAEPMDRSAMCAFPIKYVNDFFNKIVNKNNVRCLQHFYGPNHEHCFNRTLLRNSSGCEARRDEYRTEFTTALQRVDLFMGQFSEVLLTSISTFIKGDLTIANLGTSEGRFMQVVVSRSGPSTPHVNFLLDSHPVSPEVIVEHTLNQNGYTLVITGKKITKIPLNGLGCRHFQSCSQCLSAPPFVQCGWCHDKCVRSEECLSGTWTQQICLPAIYKVFPNSAPLEGGTRLTICGWDFGFRRNNKFDLKKTRVLLGNESCTLTLSESTMNTLKCTVGPAMNKHFNMSIIISNGHGTTQYSTFSYVDPVITSISPKYGPMAGGTLLTLTGNYLNSGNSRHISIGGKTCTLKSVSNSILECYTPAQTISTEFAVKLKIDLANRETSIFSYREDPIVYEIHPTKSFISGGSTITGVGKNLNSVSVPRMVINVHEAGRNFTVACQHRSNSEIICCTTPSLQQLNLQLPLKTKAFFMLDGILSKYFDLIYVHNPVFKPFEKPVMISMGNENVLEIKGNDIDPEAVKGEVLKVGNKSCENIHLHSEAVLCTVPNDLLKLNSELNIEWKQAISSTVLGKVIVQPDQNFTHHHHHH

SEQ ID NO: 44 - protein, 703 aa, synthetic construct
QRKRRNTIHEFKKSAKTTLIKIDPALKIKTKKVNTADQCANRCTRNKGLPFTCKAFVFDKARKQCLWFPFNSMSSGVKKEFGHEFDLYENKDYIRNCIIGKGRSYKGTVSITKSGIKCQPWSSMIPHEHSFLPSSYRGKDLQENYCRNPRGEEGGPWCFTSNPEVRYEVCDIPQCSEVECMTCNGESYRGLMDHTESGKICQRWDHQTPHRHKFLPERYPDKGFDDNYCRNPDGQPRPWCYTLDPHTRWEYCAIKTCADNTMNDTDVPLETTECIQGQGEGYRGTVNTIWNGIPCQRWDSQYPHEHDMTPENFKCKDLRENYCRNPDGSESPWCFTTDPNIRVGYCSQIPNCDMSHGQDCYRGNGKNYMGNLSQTRSGLTCSMWDKNMEDLHRHIFWEPDASKLNENYCRNPDDDAHGPWCYTGNPLIPWDYCPISRCEGDTTPTIVNLDHPVISCAKTKQLRVVNGIPTRTNIGWMVSLRYRNKHICGGSLIKESWVLTARQCFPSRDLKDYEAWLGIHDVHGRGDEKCKQVLNVSQLVYGPEGSDLVLMKLARPAVLDDFVSTIDLPNYGCTIPEKTSCSVYGWGYTGLINYDGLLRVAHLYIMGNEKCSQHHRGKVTLNESEICAGAEKIGSGPCEGDYGGPLVCEQHKMRMVLGVIVPGRGCAIPNRPGIFVRVAYYAKWIHKIILTYKVPQSHHHHHH

SEQ ID NO: 45 - protein, 9 aa, synthetic construct
GGGGSGGGG

SEQ ID NO: 46 - protein, 5 aa, synthetic construct
GGGGS

SEQ ID NO: 47 - protein, 227 aa, synthetic construct
DKTHTCPPCPAPELLGGPSVFLFPPKPKDTLMISRTPEVTCVVVDVSHEDPEVKFNWYVDGVEVHNAKTKPREEQYNSTYRVVSVLTVLHQDWLNGKEYKCKVSNKALPAPIEKTISKAKGQPREPQVYTLPPCREEMTKNQVSLWCLVKGFYPSDIAVEWESNGQPENNYKTTPPVLDSDGSFFLYSKLTVDKSRWQQGNVFSCSVMHEALHNHYTQKSLSLSPGK

SEQ ID NO: 48 - protein, 227 aa, synthetic construct
DKTHTCPPCPAPELLGGPSVFLFPPKPKDTLMISRTPEVTCVVVDVSHEDPEVKFNWYVDGVEVHNAKTKPREEQYNSTYRVVSVLTVLHQDWLNGKEYKCKVSNKALPAPIEKTISKAKGQPREPQVCTLPPSREEMTKNQVSLSCAVKGFYPSDIAVEWESNGQPENNYKTTPPVLDSDGSFFLVSKLTVDKSRWQQGNVFSCSVMHEALHNHYTQKSLSLSPGK

SEQ ID NO: 49 - protein, 107 aa, synthetic construct [sequence omitted]

SEQ ID NO: 50 - protein, 98 aa, synthetic construct
GIPPKIECLPIDISIDEGKVLTVASAFTGEPTPEVTWSTGGRKIHSQEQGRFHIENTDDSTTLTIKDVQKQDGGLYTLTLRNEFGSDSATVNIHIRSI

SEQ ID NO: 51 - protein, 97 aa, synthetic construct
SGAPRFLTRPKASVVSVGKDATLSCQIVGNPFPQVSWEKDKQPVTAGVRFRLAQDGDLYRLKILDLQLSDSGQYVCRARNAHGEAFACLGLQVDAEA